European Patent Application EP 4 455 279 A1, published October 30, 2024. Title: DNA POLYMERASE MUTANT AND USE THEREOF. Applicant: BGI SHENZHEN. The sequence listing filed with the application follows.

SEQUENCE LISTING (3 sequences)

SEQ ID NO: 1 - protein, 832 aa, Artificial Sequence [sequence omitted]

SEQ ID NO: 2 - protein, 832 aa, Artificial Sequence
MRGMLPLFEPKGRVLLVDGHHLAYRTFHALKGLTTSRGEPVQAVYGFAKSLLKALQEDGDTVIVVFDAKAPSFRHEAYGGYKAGRAPTPEDFPRQLALIKELVDLLGLARLEVPGYEADDVLASLAKKAEKEGYEVRILTADKDLYQLLSDRIHVLHPEGYLITPAWLWEKYGLRPDQWADYRALTGDESDNLPGVKGIGEKTARKLLEEWGSLEALLKNLDRLKPAIREKILAHMDDLKLSWDLAKVRTDLPLEVDFAKRREPDRERLRAFLERLEFGSLLHEFGLLESPKALEEAPWPPPEGAFVGFVLSRKEPMWADLLALAAARGGRVHRAPEPYKALRDLKEARGLLAKDLSVLALREGLGLPPGDDPMLLAYLLDPSNTTPEGVARRYGGEWTEEAGERAALSERLFANLWGRLEGEERLLWLYREVERPLSAVLAHMEATGVRLDVAYLRALSLEVAEEIARLEAEVFRLAGHPFNLNSRDQLERVLFDELGLPAIGKTKKTGKRSTSAAVLEALREAHPIVEKILQYRELTKLKSTYIDPLPDLIHPRTGRLHTRFNQTATATGRLSSSDPNLQNIPVRTPLGQRIRRAFIAEEGWLLVALDYSQIELRVLAHLSGDENLIRVFQEGRDIHTETASWMFGVPREAVDPLMRRAAKTINFGVLYGMSAHRLSQELAIPYEEAQAFIERYFQSFPKVRAWIEKTLEEGRRRGYVETLFGRRRYVPDLEARVKSVREAAERMAFNMPVQGTAADLMKLAMVKLFPRLEEMGARMLLQVHDELVLEAPKERAEAVARLAKEVMEGVYPLAVPLEVEVGIGEDWLSAKE

SEQ ID NO: 3 - DNA, 2499 bp, Artificial Sequence
atgcgtggcatgctgccgctgttcgagccgaagggtcgtgtgctgctggttgacggccaccacctggcgtaccgtacctttcacgcgctgaagggtctgaccaccagccgtggcgaaccggtgcaggcggtttatggtttcgcgaaaagcctgctgaaggcgctgcaagaggacggcgatacggtgatcgtggttttcgatgcgaaggcgccgagctttcgtcacgaagcgtacggtggctataaagcgggtcgtgcgccgaccccggaggactttccgcgtcaactggcgctgattaaagaactggttgatctgctgggtctggcgcgtctggaagtgccgggctacgaagcggacgatgttctggcgagcctggcgaagaaagcggagaaggaaggttacgaagtgcgtatcctgaccgcggacaaagatctgtatcagctgctgagcgaccgtatccacgttctgcacccggagggttatctgattaccccggcgtggctgtgggaaaagtacggcctgcgtccggaccaatgggcggattatcgtgcgctgaccggtgacgagagcgataacctgccgggcgttaaaggtattggcgaaaaaaccgcgcgtaagctgctggaggaatggggtagcctggaagcgctgctgaaaaacctggatcgtctgaagccggcgatccgtgagaaaattctggcgcacatggacgatctgaagctgagctgggacctggcgaaagtgcgtaccgacctgccgctggaagtggatttcgcgaagcgtcgtgagccggatcgtgaacgtctgcgtgcgttcctggagcgtctggaatttggtagcctgctgcacgagtttggcctgctggaaagcccgaaggcgctggaggaagcgccgtggccgccgccagagggtgcgttcgtgggctttgttctgagccgtaaagaaccgatgtgggcggacctgctggcgctggcggcggcgcgtggtggccgtgtgcaccgtgcgccggagccgtacaaggcgctgcgtgacctgaaagaagcgcgtggtctgctggcgaaagatctgagcgttctggcgctgcgcgaaggtctgggtctgccgccgggtgacgatccgatgctgctggcgtacctgctggatccgagcaacaccaccccggagggtgtggcgcgtcgttatggtggcgaatggaccgaggaagcgggcgagcgtgcggcgctgagcgaacgtctgttcgcgaacctgtggggtcgtctggagggcgaggaacgtctgctgtggctgtaccgtgaggtggaacgtccgctgagcgcggttctggcgcacatggaagcgaccggtgtgcgtctggacgttgcgtatctgcgtgcgctgagcctggaagtggcggaggaaatcgcgcgtctggaggcggaagttttccgtctggcgggccacccgtttaacctgaacagccgtgaccagctggagcgtgttctgtttgatgaactgggtctgccggcgattggcaagaccaaaaaaaccggcaagcgtagcaccagcgcggcggtgctggaggcgctgcgtgaagcgcacccgatcgttgagaagattctgcagtaccgtgaactgaccaagctgaaaagcacctatatcgacccgctgccggatctgattcacccgcgtaccggtcgtctgcacacccgtttcaaccaaaccgcgaccgcgaccggtcgtctgagcagcagcgacccgaacctgcagaacatcccggtgcgtaccccgctgggtcaacgtatccgtcgtgcgtttattgcggaggaaggctggctgctggttgcgctggattacagccagattgagctgcgtgttctggcgcacctgagcggtgacgaaaacctgatccgtgttttccaagagggccgtgatattcacaccgaaaccgcgagctggatgtttggtgtgccgcgtgaggcggttgacccgctgatgcgtcgtgcggcgaagaccatcaacttcggtgtgctgtatggcatgagcgcgcaccgtctgagccaggagctggcgatcccgtacgaggaagcgcaggcgtttattgaacgttatttccaaagctttccgaaggttcgtgcgtggattgagaaaaccctggaggaaggtcgtcgtcgtggttacgtggaaaccctgttcggtcgtcgtcgttacgttccggatctggaggcgcgtgtgaaaagcgttcgtgaggcggcggaacgtatggcgttcaacatgccggtgcagggtaccgcggcggacctgatgaaactggcgatggttaagctgtttccgcgtctggaggaaatgggcgcgcgtatgctgctgcaagtgcacgatgagctggttctggaagcgccgaaggagcgtgcggaagcggtggcgcgtctggcgaaagaggtgatggaaggtgtttacccgctggcggttccgctggaagttgaggtgggtatcggcgaggactggctgagcgcgaaagaataa